European Patent Application EP 4 230 637 A1, published August 23, 2023. Title: Radioconjugates of anti-HER2 antibody, and radiopharmaceuticals. Applicant: NIHON MEDI-PHYSICS CO., LTD. The sequence listing filed with the application follows.

SEQUENCE LISTING (17 sequences)

SEQ ID NO: 1 - protein, 109 aa, Homo sapiens
DIQMTQSPSSLSASVGDRVTITCRASQDVNTAVAWYQQKPGKAPKLLIYSASFLESGVPSRFSGSRSGTDFTLTISSLQPEDFATYYCQQHYTTPPTFGQGTKVEIKRT

SEQ ID NO: 2 - protein, 120 aa, Homo sapiens
EVQLVESGGGLVQPGGSLRLSCAASGFNIKDTYIHWVRQAPGKGLEWVARIYPTNGYTRYADSVKGRFTISADTSKNTAYLQMNSLRAEDTAVYYCSRWGGDGFYAMDVWGQGTLVTVSS

SEQ ID NO: 3 - protein, 13 aa, Artificial Sequence
  Peptide for modifying antibody
  SITE (6)..(6): Xaa is a lysine residue, a cysteine residue, an aspartic acid residue, a glutamic acid residue, a 2-aminosuberic acid or diaminopropionic acid.
DCAYHXGELVWCT

SEQ ID NO: 4 - protein, 17 aa, Artificial Sequence
  Peptide for modifying antibody
  SITE (8)..(8): Xaa is a lysine residue, a cysteine residue, an aspartic acid residue, a glutamic acid residue, a 2-aminosuberic acid or diaminopropionic acid.
GPDCAYHXGELVWCTFH

SEQ ID NO: 5 - protein, 13 aa, Artificial Sequence
  Peptide for modifying antibody
  SITE (6)..(6): Xaa is a lysine residue, a cysteine residue, an aspartic acid residue, a glutamic acid residue, a 2-aminosuberic acid or diaminopropionic acid.
RCAYHXGELVWCS

SEQ ID NO: 6 - protein, 17 aa, Artificial Sequence
  Peptide for modifying antibody
  SITE (8)..(8): Xaa is a lysine residue, a cysteine residue, an aspartic acid residue, a glutamic acid residue, a 2-aminosuberic acid or diaminopropionic acid.
GPRCAYHXGELVWCSFH

SEQ ID NO: 7 - protein, 17 aa, Artificial Sequence
  Peptide for modifying antibody
  SITE (8)..(8): Xaa is a lysine residue, a cysteine residue, an aspartic acid residue, a glutamic acid residue, a 2-aminosuberic acid or diaminopropionic acid.
SPDCAYHXGELVWCTFH

SEQ ID NO: 8 - protein, 17 aa, Artificial Sequence
  Peptide for modifying antibody
  SITE (8)..(8): Xaa is a lysine residue, a cysteine residue, an aspartic acid residue, a glutamic acid residue, a 2-aminosuberic acid or diaminopropionic acid.
GDDCAYHXGELVWCTFH

SEQ ID NO: 9 - protein, 17 aa, Artificial Sequence
  Peptide for modifying antibody
  SITE (8)..(8): Xaa is a lysine residue, a cysteine residue, an aspartic acid residue, a glutamic acid residue, a 2-aminosuberic acid or diaminopropionic acid.
GPSCAYHXGELVWCTFH

SEQ ID NO: 10 - protein, 17 aa, Artificial Sequence
  Peptide for modifying antibody
  SITE (8)..(8): Xaa is a lysine residue, a cysteine residue, an aspartic acid residue, a glutamic acid residue, a 2-aminosuberic acid or diaminopropionic acid.
GPDCAYHXGELVWCSFH

SEQ ID NO: 11 - protein, 17 aa, Artificial Sequence
  Peptide for modifying antibody
  SITE (8)..(8): Xaa is a lysine residue, a cysteine residue, an aspartic acid residue, a glutamic acid residue, a 2-aminosuberic acid or diaminopropionic acid.
GPDCAYHXGELVWCTHH

SEQ ID NO: 12 - protein, 17 aa, Artificial Sequence
  Peptide for modifying antibody
  SITE (8)..(8): Xaa is a lysine residue, a cysteine residue, an aspartic acid residue, a glutamic acid residue, a 2-aminosuberic acid or diaminopropionic acid.
GPDCAYHXGELVWCTFY

SEQ ID NO: 13 - protein, 17 aa, Artificial Sequence
  Peptide for modifying antibody
  SITE (8)..(8): Xaa is a lysine residue, a cysteine residue, an aspartic acid residue, a glutamic acid residue, a 2-aminosuberic acid or diaminopropionic acid.
SPDCAYHXGELVWCTFY

SEQ ID NO: 14 - protein, 17 aa, Artificial Sequence
  Peptide for modifying antibody
  SITE (8)..(8): Xaa is a lysine residue, a cysteine residue, an aspartic acid residue, a glutamic acid residue, a 2-aminosuberic acid or diaminopropionic acid.
SDDCAYHXGELVWCTFY

SEQ ID NO: 15 - protein, 17 aa, Artificial Sequence
  Peptide for modifying antibody
  SITE (8)..(8): Xaa is a lysine residue, a cysteine residue, an aspartic acid residue, a glutamic acid residue, a 2-aminosuberic acid or diaminopropionic acid.
RGNCAYHXGQLVWCTYH

SEQ ID NO: 16 - protein, 17 aa, Artificial Sequence
  Peptide for modifying antibody
  SITE (2)..(2): Xaa is a homosysteine residue.
  SITE (8)..(8): Xaa is a lysine residue, a cysteine residue, an aspartic acid residue, a glutamic acid residue, a 2-aminosuberic acid or diaminopropionic acid.
  SITE (16)..(16): Xaa is a homosysteine residue.
GXDCAYHXGELVWCTXH

SEQ ID NO: 17 - protein, 17 aa, Artificial Sequence
  Peptide for modifying antibody
  DISULFID (4)..(14)
GPDCAYHKGELVWCTFH